European Patent Specification EP 3 382 028 B1, published January 29, 2025. Title: STACKED HERBICIDE TOLERANCE EVENT 8264.44.06.1, RELATED TRANSGENIC SOYBEAN LINES, AND DETECTION THEREOF. Applicant: Dow AgroSciences LLC; M.S. Technologis, Inc. The sequence listing filed with the application follows.

SEQUENCE LISTING (29 sequences)

SEQ ID NO: 1 - DNA, 570 bp, Artificial Sequence
  5' flanking border sequence for the subject soybean Event pDAB8264.44.06.1
agcttaacatacaagtaatgtaatccacagtacgaaaaatgtgcaggttcttatttgtgctccataattgtttcttgattccgatcaaagcaagagcatccagtctcaaaattttgtcttctcaattcactcattcatcaaaatcagcagttttatgcatcaacaagcatggaatgttgaaccacccatgattaagccccatatcgttgtgttgagataactatcacctgaagttgtcttataaaaaacacatctgaatacttttataatcatacctttctcggccttttggctaagatcaagtgtagtatctgttcttatcagtttaatatctgatatgtgggtcattggcccacatgatattaaatttattttttgaagggtggggcctgacatagtagcttgctactgggggttcttaagcgtagcctgtgtcttgcactactgcatgggcctggcgcaccctacgattcagtgtatatttatgtgtgataatgtcatgggtttttattgttcttgttgtttcctctttaggaacttacatgtaaacggtaaggtcatcatggaggt

SEQ ID NO: 2 - DNA, 1499 bp, Artificial Sequence
  3' flanking border sequence for the subject soybean Event pDAB8264.44.06.1
acagagaacgaatgtcgtgtgatatgtggaacaaggcaacgacaacaacatacatgaatctcacaatagagtcggggtcgccgagttgtgatgtaatccatggcatggacatggtggccgatcgaaaaagaaaaaagaaatgcatgtatatgtgtgaaaatgagagttttttttatccaaataataaaaaaaaattaattatttacccaaaaaattatttacatgaccgatacgtacacttttttccttagttaagaaacaccgatttcttaattacatttttttatacatttagaaattggtttccttggaaccgatttcaaaatgttcattttttttttcaaaaccaagttaagaaatcggttccttggaaaacgacttcttaattgcttttttttttgttttgttttaaaattgtttgtatttttattttttttgttattaattgtctatatttgtgttctgtttaaattgaaaacaatattatttttcatatgttgttaattcttaatttcttatgcatattttatgttttatcattttttaagagttgaaatcctttgtatttttattttatttgattattataatacataattaaacaacaacttaattgaaattaaaaaatatatatttaactgacaagttgacttgaactaaaatatttaaattacaaaatagatatgaaattacaaacaatagaacaaaatatttaaatttgaaataatacaacaaaaattttaaaatacaaacaatatggcataaaattaatgttgttggcctgagcctacacaatggggggaatgcgacacatggaacatcattttggtttacctgattcttggatatccattttggtgtgtatacgagaggagacatgacaacctttagaatttcttttcatttttgggttggggcaaattcttggcttgtgacatggtgaccaacatgcttcattgcacaatttcccaagtaatcatttgtacatgttatagatacttttcagcgtatacacaagatgtatgtagttcctatactcatggtgagcatgcttataaacaacaacatgagaacaaaacatgtgcattttttgaaatttgtcacagtcacactacctttcatctagcttgaccatgaaatttctcactagttgaatctctctctccagttaattgtctcctagactaagaattgtatgtcgcattaatcgaactcaagaacaatgtgagagtttgcctttttctgtatgtctttcatagccttgtttaatacttttgtataaacttcaccaaatgtaatcactcttgcgacttctctccccctttggttgaacaatgcattacacctagtataggttgattttaccaacrcacattgccagattttgtgttttcttgagtaccaaattaattaactcagtgtccccatcgccagccaccatcccatgcgagagtccacttttcttgtggaatcttcctaagctaattaattgttagtta

SEQ ID NO: 3 - DNA, 25 bp, Artificial Sequence
  Primer 4406_WF1
aggttgtcattccgctgaagaagat

SEQ ID NO: 4 - DNA, 25 bp, Artificial Sequence
  Primer 4406_WF2
cacagtggacaattctgatttctgg

SEQ ID NO: 5 - DNA, 25 bp, Artificial Sequence
  Primer 4406_WF3
ggattgcatctgaaacggatcatat

SEQ ID NO: 6 - DNA, 25 bp, Artificial Sequence
  Primer 4406_WF4
ggaatgttgaaccacccatgattaa

SEQ ID NO: 7 - DNA, 25 bp, Artificial Sequence
  Primer 4406_WR5
catgtatgttgttgtcgttgccttg

SEQ ID NO: 8 - DNA, 25 bp, Artificial Sequence
  Primer 4406_WR6
aacattttgaaatcggttccaagga

SEQ ID NO: 9 - DNA, 25 bp, Artificial Sequence
  Primer 4406_WR7
aggctcaggccaacaacattaattt

SEQ ID NO: 10 - DNA, 27 bp, Artificial Sequence
  Primer 4406_WR8
ggagagaagtcgcaacagtgattacat

SEQ ID NO: 11 - DNA, 26 bp, Artificial Sequence
  Primer ED_v1_C1
gagtaaaggagaccgagaggatggtt

SEQ ID NO: 12 - DNA, 24 bp, Artificial Sequence
  Primer PAT_12
gaacgcttacgattggacagttga

SEQ ID NO: 13 - DNA, 10256 bp, Artificial Sequence
  Plasmid pDAB8264
agtcagcatcatcacaccaaaagttaggcccgaatagtttgaaattagaaagctcgcaattgaggtctacaggccaaattcgctcttagccgtacaatattactcaccggatcctaaccggtgtgatcatgggccgcgattaaaaatctcaattatatttggtctaatttagtttggtattgagtaaaacaaattcgaaccaaaccaaaatataaatatatagtttttatatatatgcctttaagactttttatagaattttctttaaaaaatatctagaaatatttgcgactcttctggcatgtaatatttcgttaaatatgaagtgctccatttttattaactttaaataattggttgtacgatcactttcttatcaagtgttactaaaatgcgtcaatctctttgttcttccatattcatatgtcaaaacctatcaaaattcttatatatctttttcgaatttgaagtgaaatttcgataatttaaaattaaatagaacatatcattatttaggtatcatattgatttttatacttaattactaaatttggttaactttgaaagtgtacatcaacgaaaaattagtcaaacgactaaaataaataaatatcatgtgttattaagaaaattctcctataagaatattttaatagatcatatgtttgtaaaaaaaattaatttttactaacacatatatttacttatcaaaaatttgacaaagtaagattaaaataatattcatctaacaaaaaaaaaaccagaaaatgctgaaaacccggcaaaaccgaaccaatccaaaccgatatagttggtttggtttgattttgatataaaccgaaccaactcggtccatttgcacccctaatcataatagctttaatatttcaagatattattaagttaacgttgtcaatatcctggaaattttgcaaaatgaatcaagcctatatggctgtaatatgaatttaaaagcagctcgatgtggtggtaatatgtaatttacttgattctaaaaaaatatcccaagtattaataatttctgctaggaagaaggttagctacgatttacagcaaagccagaatacaatgaaccataaagtgattgaagctcgaaatatacgaaggaacaaatatttttaaaaaaatacgcaatgacttggaacaaaagaaagtgatatattttttgttcttaaacaagcatcccctctaaagaatggcagttttcctttgcatgtaactattatgctcccttcgttacaaaaattttggactactattgggaacttcttctgaaaatagtggccaccgcttaattaaggcgcgccgacgaatgtccccgatcaaatctgagggacgttaaagcgatgataaattggaaccagaatatagaatctttgttctgctctagcttttcttctgtacattttttacgattagactatgattttcattcaataaccaaaattctgaagtttgtcatcaagttgctcaatcaaacttgtaccggtttgtttcggttttatatcagctcactgttacactttaaccaaaatcggtttatgtcttaataaaggaattgagtcggtttaactcatatccgtaccaatgcgacgtcgtgtccgcgtttcagtagctttgctcattgtcttctacgggaactttcccggacataggaaccgccctttcgttatcctcatccatcgtgaaatcaggaaataaatgttcgaagatttgaggtcaaaagtcgaatttcatgttgtctcttctatttagatacaaaattgaagcaattttcaccaatttaatgccaaaatttaaaacaacgctgataaagtgaaacttgattcgatttatatttcaaccgaaactgctgaagcaagaagaaaaagcgtaattacacataacaagaacgctaccgcaaactactaaacgccaaacccaatacaaaagtaaaacgcagacgcttaagtgagaaacccagaaaacacaaacgcggatcgggggatccactagttctagagcttaattcttgacgaaagtgctcagcacatcgaagtagtcggggaaggtcttccgggtgcacccagggtcccggatggtgacggggacctcggcacaggcggcaagggagaaagccatcgccatcctgtggtcgtcgtacgtgtcgatcgccgtcacgttcagcttctccggcggcgtgatgatgcagtagtccggcccttcctcaacagatgctcccagcttggttagctccgtccggatcgcaaccatcctctcggtctcctttactctccaggaagccacgtctctgatggctgtcgggccatcggcaaagagggcaaccacagcaagagtcatggcgacatcaggcatcttgttcatgttgacatcaatcgccttgaggtgtttcctcccaaatggctcccgcggtgggccagtaacagttacgctagtctcggtccatgtaaccttcgctcccatcatctccagtacctcagcaaacttcacatcaccctgcaaactggtggtgccacaaccttccacagtcacagtccctccagtaattgcagcaccagccaagaaatagcttgcgcttgaggcatcaccttcaacataggcatttttaggggacttgtatttttgacctcccttaatgtagaatctgtcccagctatcagaatgctctgctttcacaccaaaacgctccatcaatctcaatgtcatttcgacgtacggaatggagattaatttatcaatgatttcaatctccacatccccaagagccaaaggagcagccatcagcaaggcactcaagtactgactgctgatggagccagacagcttgaccttgccaccaggtagccctccgattccattgacacgaacaggtgggcagtcagtgccaaggaaacaatcaacatctgcaccaagctgcttcaatccgacaaccaagtcgccaatgggtctctccctcattcttggtactccatcaagcacgtaagttgcatttccaccagcagcagtaacagctgctgtcaaggaccgcattgcgattccagcattccccaagaagagctgcacttcctctttagcatcctcaactgggaactttccaccacagccaacaactacagctcttttggcagctttgtccgcttcgacagagagaccaagagtcctcaaggccccgagcatgtagtggacatcctcactgttcagcaggttatcaaccactgttgtcccctcggacagggcggcgagtaggaggatccggttggaaagcgacttggaccccggcagcttgacggtgccggagatctccttgatgggctgcagcacgatctcctcggcgccggccatgcaccggatccttccgccgttgctgacgttgccgaggcttctggaggagcggcgggcgacggggaggctggcggtggacttgagcccctggaacggagcgacggcggtggccgacgaggccatcatcacggtgggcgccatagacagcggcggcaggtacgacagcgtctcgaacttcttgttgccgtaggccggccacacctgcatacattgaactcttccaccgttgctgggaagggtggagaagtcgttagccttcttggtggtggggaaggcggcgttggacttaaggccggtgaacggagccaccatgttggcctgagcaggggcggtccggctaacggtcgcgactgaggaggagatcgaagccatggggatctgcgcatttaacaagaaattgaacagtcaattggggattttcattatccataactaaattttgaagaaattggaatactaaacgtcaccacttaaaaccctaatccagatgaatcgttatcgaaccagatataaccaaaaggggcaaaattgactcgaaaaccctagttctcgatacacggctaggtaatgacaatcgcacacagacaaatctggttatacagaacttcgaagcaagaaaaaaacgatgaagaatggatcatccaataaatcgactagactcaatcttcacaggtttatcgatccagcaaacttaaaagacggacctttattttcaaactggaatgggacaaaacccgaaactctattgtcgtaaaatcagatcgcggagacagtaacagaaaaaacattaaaaagtaatggaaagacctaaacccctgatctaattacaaacaaatcatacctgttcttcgcctgaggggttcgaaatcgataagcttggatcctctagagtcgagagaaattgatgtctgtagaagaagaagaacggttaagagtagatttgggtgagaaagatgtgaaattgtttttataggcaaagacggagagtctattttttgagcaatcagatcgcatattaaatctaacggctgagatatcgatccgtgtgtacaataaaatgatgtataaaccgtcgatctgttttaatcgacggttcatattagtgatccgcgtgatggcagtgatagccactaagaatcgtcttttgttttacatgtggcgccacaaattagggtaatgaagcggcaatattttggaactcggaaaataaaattgcgccatcacattatttgaaaattttcacatgcttttattttaaaaacccacgaattacaagttacaaccgaaaaagatttataatatagtgatttatactaattttgtagtagcttaatgtatattgatactggaaaaacaatgacaatcatatgttagtattatcaagttatcgtattgatattgatattggaacatacaatgggtattgccttctttcgaccataaatatcaccaaatttacaaagtttgtgtataccaagttatcaattgtaaatgggatgtcaacattttaatttccctttgagaaactatagaccacaagaacacacttcaatagataaagtaactatttacataagaggttttaaaatcacattaacaaaaataattaccaaccggcactcacaaatacaaacagagcacacgacatgtcaaagccacaagtaaattcgttgagtggtggtttcattacaattgtgtcacttgcagcacaaactatcttgctctgggaatcatctcagcatcaaagatcatgctcacttcaggggaacttagtgtatccatgcctcgactcatatttctcctcgacatgcatcctgcaggggcgcgccatgcccgggcaagcggccgcacaagtttgtacaaaaaagcaggctccgcggtgactgactgaaaagcttgtcgacctgcaggtcaacggatcaggatattcttgtttaagatgttgaactctatggaggtttgtatgaactgatgatctaggaccggataagttcccttcttcatagcgaacttattcaaagaatgttttgtgtatcattcttgttacattgttattaatgaaaaaatattattggtcattggactgaacacgagtgttaaatatggaccaggccccaaataagatccattgatatatgaattaaataacaagaataaatcgagtcaccaaaccacttgccttttttaacgagacttgttcaccaacttgatacaaaagtcattatcctatgcaaatcaataatcatacaaaaatatccaataacactaaaaaattaaaagaaatggataatttcacaatatgttatacgataaagaagttacttttccaagaaattcactgattttataagcccacttgcattagataaatggcaaaaaaaaacaaaaaggaaaagaaataaagcacgaagaattctagaaaatacgaaatacgcttcaatgcagtgggacccacggttcaattattgccaattttcagctccaccgtatatttaaaaaataaaacgataatgctaaaaaaatataaatcgtaacgatcgttaaatctcaacggctggatcttatgacgaccgttagaaattgtggttgtcgacgagtcagtaataaacggcgtcaaagtggttgcagccggcacacacgagtcgtgtttatcaactcaaagcacaaatacttttcctcaacctaaaaataaggcaattagccaaaaacaactttgcgtgtaaacaacgctcaatacacgtgtcattttattattagctattgcttcaccgccttagctttctcgtgacctagtcgtcctcgtcttttcttcttcttcttctataaaacaatacccaaagcttcttcttcacaattcagatttcaatttctcaaaatcttaaaaactttctctcaattctctctaccgtgatcaaggtaaatttctgtgttccttattctctcaaaatcttcgattttgttttcgttcgatcccaatttcgtatatgttctttggtttagattctgttaatcttagatcgaagacgattttctgggtttgatcgttagatatcatcttaattctcgattagggtttcataaatatcatccgatttgttcaaataatttgagttttgtcgaataattactcttcgatttgtgatttctatctagatctggtgttagtttctagtttgtgcgatcgaatttgtcgattaatctgagtttttctgattaacagagatctccatggctcagaccactctccaaatcacacccactggtgccaccttgggtgccacagtcactggtgttcaccttgccacacttgacgatgctggtttcgctgccctccatgcagcctggcttcaacatgcactcttgatcttccctgggcaacacctcagcaatgaccaacagattacctttgctaaacgctttggagcaattgagaggattggcggaggtgacattgttgccatatccaatgtcaaggcagatggcacagtgcgccagcactctcctgctgagtgggatgacatgatgaaggtcattgtgggcaacatggcctggcacgccgactcaacctacatgccagtcatggctcaaggagctgtgttcagcgcagaagttgtcccagcagttgggggcagaacctgctttgctgacatgagggcagcctacgatgcccttgatgaggcaacccgtgctcttgttcaccaaaggtctgctcgtcactcccttgtgtattctcagagcaagttgggacatgtccaacaggccgggtcagcctacataggttatggcatggacaccactgcaactcctctcagaccattggtcaaggtgcatcctgagactggaaggcccagcctcttgatcggccgccatgcccatgccatccctggcatggatgcagctgaatcagagcgcttccttgaaggacttgttgactgggcctgccaggctcccagagtccatgctcaccaatgggctgctggagatgtggttgtgtgggacaaccgctgtttgctccaccgtgctgagccctgggatttcaagttgccacgtgtgatgtggcactccagactcgctggacgcccagaaactgagggtgctgccttggtttgagtagttagcttaatcacctagagctcggtcaccagcataatttttattaatgtactaaattactgttttgttaaatgcaattttgctttctcgggattttaatatcaaaatctatttagaaatacacaatattttgttgcaggcttgctggagaatcgatctgctatcataaaaattacaaaaaaattttatttgcctcaattattttaggattggtattaaggacgcttaaattatttgtcgggtcactacgcatcattgtgattgagaagatcagcgatacgaaatattcgtagtactatcgataatttatttgaaaattcataagaaaagcaaacgttacatgaattgatgaaacaatacaaagacagataaagccacgcacatttaggatattggccgagattactgaatattgagtaagatcacggaatttctgacaggagcatgtcttcaattcagcccaaatggcagttgaaatactcaaaccgccccatatgcaggagcggatcattcattgtttgtttggttgcctttgccaacatgggagtccaaggttgcggccgcgcgccgacccagctttcttgtacaaagtggttgcggccgcttaattaaatttaaatgcccgggcgtttaaacgcggccgcttaattaaggccggcctgcagcaaacccagaaggtaattatccaagatgtagcatcaagaatccaatgtttacgggaaaaactatggaagtattatgtaagctcagcaagaagcagatcaatatgcggcacatatgcaacctatgttcaaaaatgaagaatgtacagatacaagatcctatactgccagaatacgaagaagaatacgtagaaattgaaaaagaagaaccaggcgaagaaaagaatcttgaagacgtaagcactgacgacaacaatgaaaagaagaagataaggtcggtgattgtgaaagagacatagaggacacatgtaaggtggaaaatgtaagggcggaaagtaaccttatcacaaaggaatcttatcccccactacttatccttttatatttttccgtgtcatttttgcccttgagttttcctatataaggaaccaagttcggcatttgtgaaaacaagaaaaaatttggtgtaagctattttctttgaagtactgaggatacaacttcagagaaatttgtaagtttgtagatctccatgtctccggagaggagaccagttgagattaggccagctacagcagctgatatggccgcggtttgtgatatcgttaaccattacattgagacgtctacagtgaactttaggacagagccacaaacaccacaagagtggattgatgatctagagaggttgcaagatagatacccttggttggttgctgaggttgagggtgttgtggctggtattgcttacgctgggccctggaaggctaggaacgcttacgattggacagttgagagtactgtttacgtgtcacataggcatcaaaggttgggcctaggatccacattgtacacacatttgcttaagtctatggaggcgcaaggttttaagtctgtggttgctgttataggccttccaaacgatccatctgttaggttgcatgaggctttgggatacacagcccggggtacattgcgcgcagctggatacaagcatggtggatggcatgatgttggtttttggcaaagggattttgagttgccagctcctccaaggccagttaggccagttacccagatctgaggtaccctgagcttgagcttatgagcttatgagcttagagctcggatccactagtaacggccgccagtgtgctggaattcgcccttgactagataggcgcccagatcggcggcaatagcttcttagcgccatcccgggttgatcctatctgtgttgaaatagttgcggtgggcaaggctctctttcagaaagacaggcggccaaaggaacccaaggtgaggtgggctatggctctcagttccttgtggaagcgcttggtctaaggtgcagaggtgttagcgggatgaagcaaaagtgtccgattgtaacaagatatgttgatcctacgtaaggatattaaagtatgtattcatcactaatataatcagtgtattccaatatgtactacgatttccaatgtctttattgtcgccgtatgtaatcggcgtcacaaaataatccccggtgactttcttttaatccaggatgaaataatatgttattataatttttgcgatttggtccgttataggaattgaagtgtgcttgcggtcgccaccactcccatttcataattttacatgtatttgaaaaataaaaatttatggtattcaatttaaacacgtatacttgtaaagaatgatatcttgaaagaaatatagtttaaatatttattgataaaataacaagtcaggtattatagtccaagcaaaaacataaatttattgatgcaagtttaaattcagaaatatttcaataactgattatatcagctggtacattgccgtagatgaaagactgagtgcgatattatggtgtaatacatagcggccgggtttctagtcaccggttaggatccgtttaaactcgaggctagcgcatgcacatagacacacacatcatctcattgatgcttggtaataattgtcattagattgtttttatgcatagatgcactcgaaatcagccaattttagacaagtatcaaacggatgtgacttcagtacattaaaaacgtccgcaatgtgttattaagttgtctaagcgtcaatttg

SEQ ID NO: 14 - DNA, 859 bp, Artificial Sequence
  Provides part of the 5' soybean genomic flanking and part of the 5' insert sequence
agcttaacatacaagtaatgtaatccacagtacgaaaaatgtgcaggttcttatttgtgctccataattgtttcttgattccgatcaaagcaagagcatccagtctcaaaattttgtcttctcaattcactcattcatcaaaatcagcagttttatgcatcaacaagcatggaatgttgaaccacccatgattaagccccatatcgttgtgttgagataactatcacctgaagttgtcttataaaaaacacatctgaatacttttataatcatacctttctcggccttttggctaagatcaagtgtagtatctgttcttatcagtttaatatctgatatgtgggtcattggcccacatgatattaaatttattttttgaagggtggggcctgacatagtagcttgctactgggggttcttaagcgtagcctgtgtcttgcactactgcatgggcctggcgcaccctacgattcagtgtatatttatgtgtgataatgtcatgggtttttattgttcttgttgtttcctctttaggaacttacatgtaaacggtaaggtcatcatggaggtccgaatagtttgaaattagaaagctcgcaattgaggtctacaggccaaattcgctcttagccgtacaatattactcaccggatcctaaccggtgtgatcatgggccgcgattaaaaatctcaattatatttggtctaatttagtttggtattgagtaaaacaaattcgaaccaaaccaaaatataaatatatagtttttatatatatgcctttaagactttttatagaattttctttaaaaaatatctagaaatatttgcgactcttctggcatgtaatatttcgttaa

SEQ ID NO: 15 - DNA, 1719 bp, Artificial Sequence
  Part of the 3' soybean genomic flanking and part of the 3' insert sequence
gcacatagacacacacatcatctcattgatgcttggtaataattgtcattagattgtttttatgcatagatgcactcgaaatcagccaattttagacaagtatcaaacggatgtgacttcagtacattaaaaacgtccgcaatgtgttattaagttgtctaagcgtcaatttgatttacaattgaatatatcctgccccagccagccaacagctcgatttacagagaacgaatgtcgtgtgatatgtggaacaaggcaacgacaacaacatacatgaatctcacaatagagtcggggtcgccgagttgtgatgtaatccatggcatggacatggtggccgatcgaaaaagaaaaaagaaatgcatgtatatgtgtgaaaatgagagttttttttatccaaataataaaaaaaaattaattatttacccaaaaaattatttacatgaccgatacgtacacttttttccttagttaagaaacaccgatttcttaattacatttttttatacatttagaaattggtttccttggaaccgatttcaaaatgttcattttttttttcaaaaccaagttaagaaatcggttccttggaaaacgacttcttaattgcttttttttttgttttgttttaaaattgtttgtatttttattttttttgttattaattgtctatatttgtgttctgtttaaattgaaaacaatattatttttcatatgttgttaattcttaatttcttatgcatattttatgttttatcattttttaagagttgaaatcctttgtatttttattttatttgattattataatacataattaaacaacaacttaattgaaattaaaaaatatatatttaactgacaagttgacttgaactaaaatatttaaattacaaaatagatatgaaattacaaacaatagaacaaaatatttaaatttgaaataatacaacaaaaattttaaaatacaaacaatatggcataaaattaatgttgttggcctgagcctacacaatggggggaatgcgacacatggaacatcattttggtttacctgattcttggatatccattttggtgtgtatacgagaggagacatgacaacctttagaatttcttttcatttttgggttggggcaaattcttggcttgtgacatggtgaccaacatgcttcattgcacaatttcccaagtaatcatttgtacatgttatagatacttttcagcgtatacacaagatgtatgtagttcctatactcatggtgagcatgcttataaacaacaacatgagaacaaaacatgtgcattttttgaaatttgtcacagtcacactacctttcatctagcttgaccatgaaatttctcactagttgaatctctctctccagttaattgtctcctagactaagaattgtatgtcgcattaatcgaactcaagaacaatgtgagagtttgcctttttctgtatgtctttcatagccttgtttaatacttttgtataaacttcaccaaatgtaatcactcttgcgacttctctccccctttggttgaacaatgcattacacctagtataggttgattttaccaacrcacattgccagattttgtgttttcttgagtaccaaattaattaactcagtgtccccatcgccagccaccatcccatgcgagagtccacttttcttgtggaatcttcctaagctaattaattgttagtta

SEQ ID NO: 16 - DNA, 98 bp, Artificial Sequence
  A 98 base pair sequence spanning the 5' integration junction
ttgttcttgttgtttcctctttaggaacttacatgtaaacggtaaggtcatcatggaggtccgaatagtttgaaattagaaagctcgcaattgaggtc

SEQ ID NO: 17 - DNA, 131 bp, Artificial Sequence
  A 131 base pair sequence spanning the 3' integration junction
aaacgtccgcaatgtgttattaagttgtctaagcgtcaatttgatttacaattgaatatatcctgccccagccagccaacagctcgatttacagagaacgaatgtcgtgtgatatgtggaacaaggcaacg

SEQ ID NO: 18 - DNA, 26 bp, Artificial Sequence
  Primer 4406_5'F
ttgttcttgttgtttcctctttagga

SEQ ID NO: 19 - DNA, 24 bp, Artificial Sequence
  Primer 4406_5'R
gacctcaattgcgagctttctaat

SEQ ID NO: 20 - DNA, 17 bp, Artificial Sequence
  Probe 4406_5'P
catggaggtccgaatag

SEQ ID NO: 21 - DNA, 24 bp, Artificial Sequence
  Primer 4406_3'F
aaacgtccgcaatgtgttattaag

SEQ ID NO: 22 - DNA, 22 bp, Artificial Sequence
  Primer 4406_3'R
cgttgccttgttccacatatca

SEQ ID NO: 23 - DNA, 16 bp, Artificial Sequence
  Probe 4406_3'P
acagagaacgaatgtc

SEQ ID NO: 24 - DNA, 24 bp, Artificial Sequence
  Primer GMS116F
gtaatatgggctcagaggaatggt

SEQ ID NO: 25 - DNA, 23 bp, Artificial Sequence
  Primer GMS116R
atggagaagaacattggaattgc

SEQ ID NO: 26 - DNA, 23 bp, Artificial Sequence
  Probe GMS116Probe
ccatggcccggtaccatctggtc

SEQ ID NO: 27 - DNA, 13659 bp, Artificial Sequence
  Event pDAB8264.44.06.1
ccgctgaagaagatcaagtgtgtgaaccaaagtgaaaataatgtttagaagccaacacagtggacaattttgatttctggttaatgggtgtattaaaaatatcagaaaactttcaaatatctcgagcaggcagttgggttgcctaatccatcacttgatctcaaagattcttgttgtcaagcttcgatgagtagcgaaacctaccgtgtgggctctaagctttaggttgccattgacgatcttgacacgacatatgacctatgatagcaattcaaacatggttcatatcagctgagttgcagacttagctgctagcatttcacgttgtgaatgcaagaggaaaaatacatagaaaaagagggaacaaaattgttaaccctccatatgtacaggttttagcctcaattttacccattgattgatttattattgaaaagtaatcacttatcagaaccagagtttgtaattcagcttgtatcgtaccatctaatatcttagtcaaatttgtgtataataagtatttaaatgtgagtctcttttatttaattagtttaaataattggaatacaattggcaaatgggcacttcaactataattagtgaattgatttagttgactgttatgaagtattttacttaagttagtaatagtagagtgatgtttgatgaattaaacttaagattggttgaagttattgatctcactggatccatagtttggtctgtgggattgcatctgaaacggatcatatggttttgttttgtgactgaattgtggcaatgtaacacctggactttttcacaactattgtataaatccagtatatctcacgtgaatctgaaattagtagcatgcttaacatataagtatcgatttatctaatcagtttccatatttatgaaaactgcactgttgaaaattgtgcaagcttaacatacaagtaatgtaatccacagtacgaaaaatgtgcaggttcttatttgtgctccataattgtttcttgattccgatcaaagcaagagcatccagtctcaaaattttgtcttctcaattcactcattcatcaaaatcagcagttttatgcatcaacaagcatggaatgttgaaccacccatgattaagccccatatcgttgtgttgagataactatcacctgaagttgtcttataaaaaacacatctgaatacttttataatcatacctttctcggccttttggctaagatcaagtgtagtatctgttcttatcagtttaatatctgatatgtgggtcattggcccacatgatattaaatttattttttgaagggtggggcctgacatagtagcttgctactgggggttcttaagcgtagcctgtgtcttgcactactgcatgggcctggcgcaccctacgattcagtgtatatttatgtgtgataatgtcatgggtttttattgttcttgttgtttcctctttaggaacttacatgtaaacggtaaggtcatcatggaggtccgaatagtttgaaattagaaagctcgcaattgaggtctacaggccaaattcgctcttagccgtacaatattactcaccggatcctaaccggtgtgatcatgggccgcgattaaaaatctcaattatatttggtctaatttagtttggtattgagtaaaacaaattcgaaccaaaccaaaatataaatatatagtttttatatatatgcctttaagactttttatagaattttctttaaaaaatatctagaaatatttgcgactcttctggcatgtaatatttcgttaaatatgaagtgctccatttttattaactttaaataattggttgtacgatcactttcttatcaagtgttactaaaatgcgtcaatctctttgttcttccatattcatatgtcaaaacctatcaaaattcttatatatctttttcgaatttgaagtgaaatttcgataatttaaaattaaatagaacatatcattatttaggtatcatattgatttttatacttaattactaaatttggttaactttgaaagtgtacatcaacgaaaaattagtcaaacgactaaaataaataaatatcatgtgttattaagaaaattctcctataagaatattttaatagatcatatgtttgtaaaaaaaattaatttttactaacacatatatttacttatcaaaaatttgacaaagtaagattaaaataatattcatctaacaaaaaaaaaaccagaaaatgctgaaaacccggcaaaaccgaaccaatccaaaccgatatagttggtttggtttgattttgatataaaccgaaccaactcggtccatttgcacccctaatcataatagctttaatatttcaagatattattaagttaacgttgtcaatatcctggaaattttgcaaaatgaatcaagcctatatggctgtaatatgaatttaaaagcagctcgatgtggtggtaatatgtaatttacttgattctaaaaaaatatcccaagtattaataatttctgctaggaagaaggttagctacgatttacagcaaagccagaatacaatgaaccataaagtgattgaagctcgaaatatacgaaggaacaaatatttttaaaaaaatacgcaatgacttggaacaaaagaaagtgatatattttttgttcttaaacaagcatcccctctaaagaatggcagttttcctttgcatgtaactattatgctcccttcgttacaaaaattttggactactattgggaacttcttctgaaaatagtggccaccgcttaattaaggcgcgccgacgaatgtccccgatcaaatctgagggacgttaaagcgatgataaattggaaccagaatatagaatctttgttctgctctagcttttcttctgtacattttttacgattagactatgattttcattcaataaccaaaattctgaagtttgtcatcaagttgctcaatcaaacttgtaccggtttgtttcggttttatatcagctcactgttacactttaaccaaaatcggtttatgtcttaataaaggaattgagtcggtttaactcatatccgtaccaatgcgacgtcgtgtccgcgtttcagtagctttgctcattgtcttctacgggaactttcccggacataggaaccgccctttcgttatcctcatccatcgtgaaatcaggaaataaatgttcgaagatttgaggtcaaaagtcgaatttcatgttgtctcttctatttagatacaaaattgaagcaattttcaccaatttaatgccaaaatttaaaacaacgctgataaagtgaaacttgattcgatttatatttcaaccgaaactgctgaagcaagaagaaaaagcgtaattacacataacaagaacgctaccgcaaactactaaacgccaaacccaatacaaaagtaaaacgcagacgcttaagtgagaaacccagaaaacacaaacgcggatcgggggatccactagttctagagcttaattcttgacgaaagtgctcagcacatcgaagtagtcggggaaggtcttccgggtgcacccagggtcccggatggtgacggggacctcggcacaggcggcaagggagaaagccatcgccatcctgtggtcgtcgtacgtgtcgatcgccgtcacgttcagcttctccggcggcgtgatgatgcagtagtccggcccttcctcaacagatgctcccagcttggttagctccgtccggatcgcaaccatcctctcggtctcctttactctccaggaagccacgtctctgatggctgtcgggccatcggcaaagagggcaaccacagcaagagtcatggcgacatcaggcatcttgttcatgttgacatcaatcgccttgaggtgtttcctcccaaatggctcccgcggtgggccagtaacagttacgctagtctcggtccatgtaaccttcgctcccatcatctccagtacctcagcaaacttcacatcaccctgcaaactggtggtgccacaaccttccacagtcacagtccctccagtaattgcagcaccagccaagaaatagcttgcgcttgaggcatcaccttcaacataggcatttttaggggacttgtatttttgacctcccttaatgtagaatctgtcccagctatcagaatgctctgctttcacaccaaaacgctccatcaatctcaatgtcatttcgacgtacggaatggagattaatttatcaatgatttcaatctccacatccccaagagccaaaggagcagccatcagcaaggcactcaagtactgactgctgatggagccagacagcttgaccttgccaccaggtagccctccgattccattgacacgaacaggtgggcagtcagtgccaaggaaacaatcaacatctgcaccaagctgcttcaatccgacaaccaagtcgccaatgggtctctccctcattcttggtactccatcaagcacgtaagttgcatttccaccagcagcagtaacagctgctgtcaaggaccgcattgcgattccagcattccccaagaagagctgcacttcctctttagcatcctcaactgggaactttccaccacagccaacaactacagctcttttggcagctttgtccgcttcgacagagagaccaagagtcctcaaggccccgagcatgtagtggacatcctcactgttcagcaggttatcaaccactgttgtcccctcggacagggcggcgagtaggaggatccggttggaaagcgacttggaccccggcagcttgacggtgccggagatctccttgatgggctgcagcacgatctcctcggcgccggccatgcaccggatccttccgccgttgctgacgttgccgaggcttctggaggagcggcgggcgacggggaggctggcggtggacttgagcccctggaacggagcgacggcggtggccgacgaggccatcatcacggtgggcgccatagacagcggcggcaggtacgacagcgtctcgaacttcttgttgccgtaggccggccacacctgcatacattgaactcttccaccgttgctgggaagggtggagaagtcgttagccttcttggtggtggggaaggcggcgttggacttaaggccggtgaacggagccaccatgttggcctgagcaggggcggtccggctaacggtcgcgactgaggaggagatcgaagccatggggatctgcgcatttaacaagaaattgaacagtcaattggggattttcattatccataactaaattttgaagaaattggaatactaaacgtcaccacttaaaaccctaatccagatgaatcgttatcgaaccagatataaccaaaaggggcaaaattgactcgaaaaccctagttctcgatacacggctaggtaatgacaatcgcacacagacaaatctggttatacagaacttcgaagcaagaaaaaaacgatgaagaatggatcatccaataaatcgactagactcaatcttcacaggtttatcgatccagcaaacttaaaagacggacctttattttcaaactggaatgggacaaaacccgaaactctattgtcgtaaaatcagatcgcggagacagtaacagaaaaaacattaaaaagtaatggaaagacctaaacccctgatctaattacaaacaaatcatacctgttcttcgcctgaggggttcgaaatcgataagcttggatcctctagagtcgagagaaattgatgtctgtagaagaagaagaacggttaagagtagatttgggtgagaaagatgtgaaattgtttttataggcaaagacggagagtctattttttgagcaatcagatcgcatattaaatctaacggctgagatatcgatccgtgtgtacaataaaatgatgtataaaccgtcgatctgttttaatcgacggttcatattagtgatccgcgtgatggcagtgatagccactaagaatcgtcttttgttttacatgtggcgccacaaattagggtaatgaagcggcaatattttggaactcggaaaataaaattgcgccatcacattatttgaaaattttcacatgcttttattttaaaaacccacgaattacaagttacaaccgaaaaagatttataatatagtgatttatactaattttgtagtagcttaatgtatattgatactggaaaaacaatgacaatcatatgttagtattatcaagttatcgtattgatattgatattggaacatacaatgggtattgccttctttcgaccataaatatcaccaaatttacaaagtttgtgtataccaagttatcaattgtaaatgggatgtcaacattttaatttccctttgagaaactatagaccacaagaacacacttcaatagataaagtaactatttacataagaggttttaaaatcacattaacaaaaataattaccaaccggcactcacaaatacaaacagagcacacgacatgtcaaagccacaagtaaattcgttgagtggtggtttcattacaattgtgtcacttgcagcacaaactatcttgctctgggaatcatctcagcatcaaagatcatgctcacttcaggggaacttagtgtatccatgcctcgactcatatttctcctcgacatgcatcctgcaggggcgcgccatgcccgggcaagcggccgcacaagtttgtacaaaaaagcaggctccgcggtgactgactgaaaagcttgtcgacctgcaggtcaacggatcaggatattcttgtttaagatgttgaactctatggaggtttgtatgaactgatgatctaggaccggataagttcccttcttcatagcgaacttattcaaagaatgttttgtgtatcattcttgttacattgttattaatgaaaaaatattattggtcattggactgaacacgagtgttaaatatggaccaggccccaaataagatccattgatatatgaattaaataacaagaataaatcgagtcaccaaaccacttgccttttttaacgagacttgttcaccaacttgatacaaaagtcattatcctatgcaaatcaataatcatacaaaaatatccaataacactaaaaaattaaaagaaatggataatttcacaatatgttatacgataaagaagttacttttccaagaaattcactgattttataagcccacttgcattagataaatggcaaaaaaaaacaaaaaggaaaagaaataaagcacgaagaattctagaaaatacgaaatacgcttcaatgcagtgggacccacggttcaattattgccaattttcagctccaccgtatatttaaaaaataaaacgataatgctaaaaaaatataaatcgtaacgatcgttaaatctcaacggctggatcttatgacgaccgttagaaattgtggttgtcgacgagtcagtaataaacggcgtcaaagtggttgcagccggcacacacgagtcgtgtttatcaactcaaagcacaaatacttttcctcaacctaaaaataaggcaattagccaaaaacaactttgcgtgtaaacaacgctcaatacacgtgtcattttattattagctattgcttcaccgccttagctttctcgtgacctagtcgtcctcgtcttttcttcttcttcttctataaaacaatacccaaagcttcttcttcacaattcagatttcaatttctcaaaatcttaaaaactttctctcaattctctctaccgtgatcaaggtaaatttctgtgttccttattctctcaaaatcttcgattttgttttcgttcgatcccaatttcgtatatgttctttggtttagattctgttaatcttagatcgaagacgattttctgggtttgatcgttagatatcatcttaattctcgattagggtttcataaatatcatccgatttgttcaaataatttgagttttgtcgaataattactcttcgatttgtgatttctatctagatctggtgttagtttctagtttgtgcgatcgaatttgtcgattaatctgagtttttctgattaacagagatctccatggctcagaccactctccaaatcacacccactggtgccaccttgggtgccacagtcactggtgttcaccttgccacacttgacgatgctggtttcgctgccctccatgcagcctggcttcaacatgcactcttgatcttccctgggcaacacctcagcaatgaccaacagattacctttgctaaacgctttggagcaattgagaggattggcggaggtgacattgttgccatatccaatgtcaaggcagatggcacagtgcgccagcactctcctgctgagtgggatgacatgatgaaggtcattgtgggcaacatggcctggcacgccgactcaacctacatgccagtcatggctcaaggagctgtgttcagcgcagaagttgtcccagcagttgggggcagaacctgctttgctgacatgagggcagcctacgatgcccttgatgaggcaacccgtgctcttgttcaccaaaggtctgctcgtcactcccttgtgtattctcagagcaagttgggacatgtccaacaggccgggtcagcctacataggttatggcatggacaccactgcaactcctctcagaccattggtcaaggtgcatcctgagactggaaggcccagcctcttgatcggccgccatgcccatgccatccctggcatggatgcagctgaatcagagcgcttccttgaaggacttgttgactgggcctgccaggctcccagagtccatgctcaccaatgggctgctggagatgtggttgtgtgggacaaccgctgtttgctccaccgtgctgagccctgggatttcaagttgccacgtgtgatgtggcactccagactcgctggacgcccagaaactgagggtgctgccttggtttgagtagttagcttaatcacctagagctcggtcaccagcataatttttattaatgtactaaattactgttttgttaaatgcaattttgctttctcgggattttaatatcaaaatctatttagaaatacacaatattttgttgcaggcttgctggagaatcgatctgctatcataaaaattacaaaaaaattttatttgcctcaattattttaggattggtattaaggacgcttaaattatttgtcgggtcactacgcatcattgtgattgagaagatcagcgatacgaaatattcgtagtactatcgataatttatttgaaaattcataagaaaagcaaacgttacatgaattgatgaaacaatacaaagacagataaagccacgcacatttaggatattggccgagattactgaatattgagtaagatcacggaatttctgacaggagcatgtcttcaattcagcccaaatggcagttgaaatactcaaaccgccccatatgcaggagcggatcattcattgtttgtttggttgcctttgccaacatgggagtccaaggttgcggccgcgcgccgacccagctttcttgtacaaagtggttgcggccgcttaattaaatttaaatgcccgggcgtttaaacgcggccgcttaattaaggccggcctgcagcaaacccagaaggtaattatccaagatgtagcatcaagaatccaatgtttacgggaaaaactatggaagtattatgtaagctcagcaagaagcagatcaatatgcggcacatatgcaacctatgttcaaaaatgaagaatgtacagatacaagatcctatactgccagaatacgaagaagaatacgtagaaattgaaaaagaagaaccaggcgaagaaaagaatcttgaagacgtaagcactgacgacaacaatgaaaagaagaagataaggtcggtgattgtgaaagagacatagaggacacatgtaaggtggaaaatgtaagggcggaaagtaaccttatcacaaaggaatcttatcccccactacttatccttttatatttttccgtgtcatttttgcccttgagttttcctatataaggaaccaagttcggcatttgtgaaaacaagaaaaaatttggtgtaagctattttctttgaagtactgaggatacaacttcagagaaatttgtaagtttgtagatctccatgtctccggagaggagaccagttgagattaggccagctacagcagctgatatggccgcggtttgtgatatcgttaaccattacattgagacgtctacagtgaactttaggacagagccacaaacaccacaagagtggattgatgatctagagaggttgcaagatagatacccttggttggttgctgaggttgagggtgttgtggctggtattgcttacgctgggccctggaaggctaggaacgcttacgattggacagttgagagtactgtttacgtgtcacataggcatcaaaggttgggcctaggatccacattgtacacacatttgcttaagtctatggaggcgcaaggttttaagtctgtggttgctgttataggccttccaaacgatccatctgttaggttgcatgaggctttgggatacacagcccggggtacattgcgcgcagctggatacaagcatggtggatggcatgatgttggtttttggcaaagggattttgagttgccagctcctccaaggccagttaggccagttacccagatctgaggtaccctgagcttgagcttatgagcttatgagcttagagctcggatccactagtaacggccgccagtgtgctggaattcgcccttgactagataggcgcccagatcggcggcaatagcttcttagcgccatcccgggttgatcctatctgtgttgaaatagttgcggtgggcaaggctctctttcagaaagacaggcggccaaaggaacccaaggtgaggtgggctatggctctcagttccttgtggaagcgcttggtctaaggtgcagaggtgttagcgggatgaagcaaaagtgtccgattgtaacaagatatgttgatcctacgtaaggatattaaagtatgtattcatcactaatataatcagtgtattccaatatgtactacgatttccaatgtctttattgtcgccgtatgtaatcggcgtcacaaaataatccccggtgactttcttttaatccaggatgaaataatatgttattataatttttgcgatttggtccgttataggaattgaagtgtgcttgcggtcgccaccactcccatttcataattttacatgtatttgaaaaataaaaatttatggtattcaatttaaacacgtatacttgtaaagaatgatatcttgaaagaaatatagtttaaatatttattgataaaataacaagtcaggtattatagtccaagcaaaaacataaatttattgatgcaagtttaaattcagaaatatttcaataactgattatatcagctggtacattgccgtagatgaaagactgagtgcgatattatggtgtaatacatagcggccgggtttctagtcaccggttaggatccgtttaaactcgaggctagcgcatgcacatagacacacacatcatctcattgatgcttggtaataattgtcattagattgtttttatgcatagatgcactcgaaatcagccaattttagacaagtatcaaacggatgtgacttcagtacattaaaaacgtccgcaatgtgttattaagttgtctaagcgtcaatttgatttacaattgaatatatcctgccccagccagccaacagctcgatttacagagaacgaatgtcgtgtgatatgtggaacaaggcaacgacaacaacatacatgaatctcacaatagagtcggggtcgccgagttgtgatgtaatccatggcatggacatggtggccgatcgaaaaagaaaaaagaaatgcatgtatatgtgtgaaaatgagagttttttttatccaaataataaaaaaaaattaattatttacccaaaaaattatttacatgaccgatacgtacacttttttccttagttaagaaacaccgatttcttaattacatttttttatacatttagaaattggtttccttggaaccgatttcaaaatgttcattttttttttcaaaaccaagttaagaaatcggttccttggaaaacgacttcttaattgcttttttttttgttttgttttaaaattgtttgtatttttattttttttgttattaattgtctatatttgtgttctgtttaaattgaaaacaatattatttttcatatgttgttaattcttaatttcttatgcatattttatgttttatcattttttaagagttgaaatcctttgtatttttattttatttgattattataatacataattaaacaacaacttaattgaaattaaaaaatatatatttaactgacaagttgacttgaactaaaatatttaaattacaaaatagatatgaaattacaaacaatagaacaaaatatttaaatttgaaataatacaacaaaaattttaaaatacaaacaatatggcataaaattaatgttgttggcctgagcctacacaatggggggaatgcgacacatggaacatcattttggtttacctgattcttggatatccattttggtgtgtatacgagaggagacatgacaacctttagaatttcttttcatttttgggttggggcaaattcttggcttgtgacatggtgaccaacatgcttcattgcacaatttcccaagtaatcatttgtacatgttatagatacttttcagcgtatacacaagatgtatgtagttcctatactcatggtgagcatgcttataaacaacaacatgagaacaaaacatgtgcattttttgaaatttgtcacagtcacactacctttcatctagcttgaccatgaaatttctcactagttgaatctctctctccagttaattgtctcctagactaagaattgtatgtcgcattaatcgaactcaagaacaatgtgagagtttgcctttttctgtatgtctttcatagccttgtttaatacttttgtataaacttcaccaaatgtaatcactcttgcgacttctctccccctttggttgaacaatgcattacacctagtataggttgattttaccaacacacattgccagattttgtgttttcttgagtaccaaattaattaactcagtgtccccatcgccagccaccatcccatgcgagagtccacttttcttgtggaatcttcctaagctaattaattgttagttcagcttggccttaaaacacacatgacaaatatttttattataaaacaaacacccagtgatacaacaatgaacaacacacatgacaactacaaatcattaaataatacaattacaatcaaataatttggggagggggtcttcaaaacttgattcaaggttcattgtatcatcgaggtattcacccaaaccctccaaattcaaagagcttgcagaaactggtggtggttgtgcatatgtttatgtgggtgtgtctacggtgataacataaaactcaaggcatgtgaagttgaagagtttcccaaatatagaaaacatagtaattatttcctcatcatcttgcagcatacatgccctgtactgaaaacaatcaccaacaaatgatacgggaca

SEQ ID NO: 28 - DNA, 14619 bp, Artificial
  Hypothetical sequence of Event 9582.812.9.1 containing 5' genomic flank, 9582 T-strand insert, 3' genomic flank
ttaattataatgactttattataaaatgaacaatttcaaaatcttcacactccaattttagattccttttatatcattttctattgagtaaaccaccatttccattcttaaaaatgtgaggcctcgcataaaagcatgaaaatggcaaaaacatccccaaaattacattttatcagtccagttaatcaatcgtaaggatcttagtgtctctattaacatatgatgaggtgacgtgttaagtgttatgccatgtacttgttgatctgtcatgttgcgatcacgtcagcataaatcaaaataaaacttttaaagtacaaaatgataataatattttatttatttatttcctctcgcatcccaagatgacagtgaagaaaataattttttgagaccgataattctaacatacactattgacttcagattataaagtactgttcaaatatgaaatttaaatgctattctagaccaaaatctgaaaattaccaaaatttccctcatgcatcaaactatattgaatctcattttaagacaaaatacaattggaaaaattataaaagctttattttaaacttagaaaattactataatatttgaatttttttctacaactatctagatttttgtttaaaattatcaaaataccctgagccttttgatcaagagtattattgtctttagttattgtcgaaaatattatcaattgacagtataagtttagtcactattttgattaaatattatactttttttaaggattaattattatacttttataacttaatcctttttattataaaatgaacaattttaaaatcttctcactccaattttatactcactttatattcttaataatatgttgtatgagcagaactaaactgaaattccttaaaaagaaagtcttgatattggtatgagtcttgtgaataaaagaattgattgagggattccactaaatcttgccactgactttttatcattgtctatttttgtttcagaaatcaaatcagtatatatacttttttatctgtccattgttcaatttcgagcgtctcgatatattatgcgcctaaattggacatccgagttaaaagttatgaccattcgaatttcccgacacccagtcagcatcatcacaccaaaagttaggcccgaatagtttgaaattagaaagctcgcaattgaggtctacaggccaaattcgctcttagccgtacaatattactcaccggatcctaaccggtgtgatcatgggccgcgattaaaaatctcaattatatttggtctaatttagtttggtattgagtaaaacaaattcggcgccatgcccgggcaagcggccgcacaagtttgtacaaaaaagcaggctccgcggtgactgactgaaaagcttgtcgacctgcaggtcaacggatcaggatattcttgtttaagatgttgaactctatggaggtttgtatgaactgatgatctaggaccggataagttcccttcttcatagcgaacttattcaaagaatgttttgtgtatcattcttgttacattgttattaatgaaaaaatattattggtcattggactgaacacgagtgttaaatatggaccaggccccaaataagatccattgatatatgaattaaataacaagaataaatcgagtcaccaaaccacttgccttttttaacgagacttgttcaccaacttgatacaaaagtcattatcctatgcaaatcaataatcatacaaaaatatccaataacactaaaaaattaaaagaaatggataatttcacaatatgttatacgataaagaagttacttttccaagaaattcactgattttataagcccacttgcattagataaatggcaaaaaaaaacaaaaaggaaaagaaataaagcacgaagaattctagaaaatacgaaatacgcttcaatgcagtgggacccacggttcaattattgccaattttcagctccaccgtatatttaaaaaataaaacgataatgctaaaaaaatataaatcgtaacgatcgttaaatctcaacggctggatcttatgacgaccgttagaaattgtggttgtcgacgagtcagtaataaacggcgtcaaagtggttgcagccggcacacacgagtcgtgtttatcaactcaaagcacaaatacttttcctcaacctaaaaataaggcaattagccaaaaacaactttgcgtgtaaacaacgctcaatacacgtgtcattttattattagctattgcttcaccgccttagctttctcgtgacctagtcgtcctcgtcttttcttcttcttcttctataaaacaatacccaaagcttcttcttcacaattcagatttcaatttctcaaaatcttaaaaactttctctcaattctctctaccgtgatcaaggtaaatttctgtgttccttattctctcaaaatcttcgattttgttttcgttcgatcccaatttcgtatatgttctttggtttagattctgttaatcttagatcgaagacgattttctgggtttgatcgttagatatcatcttaattctcgattagggtttcataaatatcatccgatttgttcaaataatttgagttttgtcgaataattactcttcgatttgtgatttctatctagatctggtgttagtttctagtttgtgcgatcgaatttgtcgattaatctgagtttttctgattaacagagatctccatggagaacaatatccagaaccagtgtgtcccatacaattgcctcaacaatcctgaagttgagatcctcaacgaagagaggagcactggacgccttccccttgacatctccctctccctcacaaggttccttttgtctgagtttgttcctggtgtgggtgtggcctttggcctctttgacctcatctggggcttcatcaccccatctgattggagcctcttccttctccagattgaacaattgattgagcagaggattgagacccttgaaaggaacagagccatcaccacacttcgtggccttgctgacagctatgaaatctacattgaagcactccgtgagtgggaagccaatcccaacaatgctcaactccgtgaagatgtgaggattcgctttgccaacacagatgacgctttgatcacagccatcaacaatttcaccctcaccagctttgagatccctttgctctcagtctatgttcaagctgcaaacctccacttgagcttgcttagggatgctgtgtccttcggacaaggttggggacttgacatagccactgtcaacaatcactacaacagactcatcaacttgattcatcgctacaccaaacattgcttggacacctacaatcaaggattggagaacctcagaggcaccaacactcgccaatgggcaaggttcaaccagtttagaagggatctcacactcactgtgcttgacatagttgctctcttccccaactatgatgttcgcacctacccaattcaaaccagctcccaacttacaagggaaatctacacctcctcagtcattgaggacagcccagtttctgccaacatacccaatggtttcaaccgtgctgagtttggtgtcagaccaccccatctcatggacttcatgaactccttgtttgtgactgccgagactgttaggtcccaaactgtgtggggaggccaccttgttagctcccgcaacaccgctggcaaccgcatcaacttcccatcctatggggttttcaatcctggtggagccatctggattgcagatgaggacccaaggcctttctacagaaccttgtcagatcctgtctttgtcagaggaggctttggcaatccacactatgttcttggtttgaggggagtggcttttcagcagactggcaccaatcacacccgcacattcagaaacagcggcaccattgacagccttgatgagatcccacctcaagacaacagcggagcaccctggaacgactactcccatgtgctcaatcatgtcacctttgtgcgctggcctggtgagatcagcggttcagattcttggagagcaccaatgttctcatggacccatcgctctgccacacccacaaacaccattgatccagagagaatcacccagattcccttggtgaaggcacacacacttcagtctggaaccacagttgtcagagggcctgggttcactggtggagacattctcagacgcacctctggagggccatttgcttacaccattgtcaacatcaatgggcaacttccccagcgttaccgtgccagaatccgctatgcttccaccactaacttgagaatctatgtcacagttgctggtgaaaggatctttgctggtcagttcaacaagacaatggacactggtgatccattgacattccagtcattctcctatgccaccatcaacactgcattcacctttccaatgagccagtccagcttcacagtgggtgcagataccttcagctccggcaatgaggtgtacattgaccgctttgagttgattccagtgactgccacacttgaggctgagtctgacttggagcgtgctcagaaggccgtgaatgctctcttcacctcttcaaatcagattgggctcaagacagatgtgactgactaccatatagaccgtgtttccaatcttgttgagtgcctctctgatgagttctgcttggatgagaagaaagagttgtcagagaaggtcaagcacgccaagaggctctctgatgagaggaacttgcttcaagatcccaacttcagagggatcaaccgtcaattggatcgtggatggaggggatcaactgacataaccattcaaggaggtgacgatgtgttcaaggagaactatgtcacactcttggggacctttgatgagtgctacccaacatacctttaccagaagatagacgaaagcaagctcaaggcctacacaagataccagttgagaggttacattgaggactctcaagaccttgaaatctacctcatcagatacaacgccaaacatgagacagtcaatgtgcctgggactggttcactctggccactttcagccccaagccccattggcaagtgtgcccatcactcacatcacttctccttggacatagatgttggctgcactgacttgaatgaggaccttggtgtgtgggtgatcttcaagatcaagacccaagatggccatgcaaggttgggcaatcttgagtttcttgaagagaaaccacttgttggagaagcccttgccagagtgaagagggctgagaagaaatggagggacaagagagagaagttggagtgggaaacaaacattgtgtacaaagaagccaaagaatcagttgatgctttgtttgtgaactcccaatatgataggctccaagctgacaccaacatagcaatgattcatgctgcagacaaaagggttcacagcattcgtgaagcataccttcctgaactctcagtgattcctggggtcaatgctgcaatctttgaagagcttgaaggacgcatcttcactgccttctccttgtatgatgcaaggaatgtcatcaagaatggtgacttcaacaatggcctttcctgctggaatgtgaaagggcacgtggatgttgaagagcagaacaatcaccgctctgtccttgttgtccctgagtgggaagctgaagtttcacaagaagttcgtgtctgccctggtcgtggctacattcttcgtgtgactgcttacaaagaaggctatggagaaggttgtgtcaccatccacgagatagagaacaatactgatgaattgaagttcagcaactgtgttgaggaagaggtctacccaaacaatactgtcacttgcaatgactacactgcaactcaagaagagtatgagggcacttacacttctcgcaaccgtggctatgatggagcctatgagagcaactcatctgtgcctgctgactatgcttcagcctatgaagagaaggcatacactgatggaaggcgtgacaatccttgtgaaagcaacagaggctatggggactacacacccctcccagctggctatgtgaccaaagagttggagtactttcctgaaactgacaaggtttggattgagataggagaaactgaaggcacattcatagttgactctgtggagcttttgctcatggaagagtgagtagttagcttaatcacctagagctcggtcaccagcataatttttattaatgtactaaattactgttttgttaaatgcaattttgctttctcgggattttaatatcaaaatctatttagaaatacacaatattttgttgcaggcttgctggagaatcgatctgctatcataaaaattacaaaaaaattttatttgcctcaattattttaggattggtattaaggacgcttaaattatttgtcgggtcactacgcatcattgtgattgagaagatcagcgatacgaaatattcgtagtactatcgataatttatttgaaaattcataagaaaagcaaacgttacatgaattgatgaaacaatacaaagacagataaagccacgcacatttaggatattggccgagattactgaatattgagtaagatcacggaatttctgacaggagcatgtcttcaattcagcccaaatggcagttgaaatactcaaaccgccccatatgcaggagcggatcattcattgtttgtttggttgcctttgccaacatgggagtccaaggttgcggccgcgcgccgaaaacaactttgtatacaaaagttgccgcggtgactgactgaactaaacccagaaggtaattatccaagatgtagcatcaagaatccaatgtttacgggaaaaactatggaagtattatgtaagctcagcaagaagcagatcaatatgcggcacatatgcaacctatgttcaaaaatgaagaatgtacagatacaagatcctatactgccagaatacgaagaagaatacgtagaaattgaaaaagaagaaccaggcgaagaaaagaatcttgaagacgtaagcactgacgacaacaatgaaaagaagaagataaggtcggtgattgtgaaagagacatagaggacacatgtaaggtggaaaatgtaagggcggaaagtaaccttatcacaaaggaatcttatcccccactacttatccttttatatttttccgtgtcatttttgcccttgagttttcctatataaggaaccaagttcggcatttgtgaaaacaagaaaaaatttggtgtaagctattttctttgaagtactgaggatacaacttcagagaaatttgtaagtttgtagatccaacaatggacaacaatcccaacatcaacgagtgcattccttacaactgcctgagcaaccctgaggttgaggtgctgggtggagaacggattgagactggttacacacctatcgacatctcgttgtcacttacccaattccttttgtcagagttcgtgcccggtgctggattcgtgcttggacttgtcgatatcatttggggaatctttggtccctctcaatgggacgcctttcttgtacagatagagcagttaattaaccaaagaatagaagaattcgctaggaaccaagccatctcaaggttagaaggcctcagcaacctttaccagatttacgcagaatcttttcgagagtgggaagcagacccgaccaatcctgccttaagagaggagatgcgcattcaattcaatgacatgaacagcgcgctgacgaccgcaattccgctcttcgccgttcagaattaccaagttcctcttttatccgtgtacgtgcaggctgccaacctgcacttgtcggtgctccgcgatgtctccgtgttcggacaacggtggggctttgatgccgcaactatcaatagtcgttataatgatctgactaggcttattggcaactataccgattatgctgttcgctggtacaacacgggtctcgaacgtgtctggggaccggattctagagattgggtcaggtacaaccagttcaggcgagagttgacactaactgtcctagacattgtcgctctctttcccaactacgactctaggcgctacccaatccgtactgtgtcacaattgacccgggaaatctacacaaacccagtcctcgagaacttcgacggtagctttcgaggctcggctcagggcatagagagaagcatcaggtctccacacctgatggacatattgaacagtatcacgatctacaccgatgcgcaccgcggttattactactggtcagggcatcagatcatggcatcacccgttgggttctctggaccagaattcactttcccactttacgggactatgggcaatgcagctccacaacaacgtattgttgctcaactcggtcagggcgtgtatagaaccttgtccagcactctatataggagacctttcaacatcggcatcaacaatcaacaattgtctgtgcttgacgggacagaatttgcctatggaacctcctcaaatctgccatccgctgtctacagaaagagcggaacagttgatagcttggatgagatccctccacagaacaacaacgttccacctaggcaagggtttagccatcgccttagccatgtgtccatgttccgttcaggctttagtaatagcagcgttagtatcatcagagctccgatgttctcttggatacatcgtagtgctgagtttaacaacataattgcatccgatagcattactcagatcccagctgtcaaggggaactttctctttaatggttctgtcatttcaggaccaggattcactggaggcgacttggttaggctgaattcttccggcaacaacatccagaatagagggtatattgaagtgcccattcacttcccatcgacatctaccagatatcgtgttcgtgtaaggtatgcctctgttacccctattcacctcaacgtcaattggggtaattcctccatcttttccaatacagtaccagcgacagctacatccttggataatctccaatctagcgatttcggttacttcgaaagtgccaatgccttcacctcttccctaggtaacatagtaggtgttagaaatttctccggaaccgccggagtgataatcgaccgcttcgaattcattcccgttactgcaacgctcgaggcagagtctgacttggaaagagcacagaaggcggtgaatgctctgttcacttcgtccaatcagattgggctcaagacagatgtgactgactatcacatcgatcgcgtttccaaccttgttgagtgcctctctgatgagttctgtttggatgagaagaaggagttgtccgagaaggtcaaacatgctaagcgacttagtgatgagcggaacttgcttcaagatcccaactttcgcgggatcaacaggcaactagatcgtggatggaggggaagtacggacatcaccattcaaggaggtgatgatgtgttcaaggagaactatgttacgctcttgggtacctttgatgagtgctatccaacatacctgtaccagaagatagatgaatcgaaactcaaagcctacacaagataccagttgagaggttacatcgaggacagtcaagaccttgagatctacctcatcagatacaacgccaaacatgagacagtcaatgtgcctgggacgggttcactctggccactttcagccccaagtcccatcggcaagtgtgcccatcactcacaccacttctccttggacatagacgttggctgtaccgacctgaacgaagacctcggtgtgtgggtgatcttcaagatcaagactcaagatggccatgccaggctaggcaatctggagtttctagaagagaaaccacttgttggagaagccctcgctagagtgaagagggctgagaagaagtggagggacaagagagagaagttggaatgggaaacaaacattgtgtacaaagaagccaaagaaagcgttgacgctctgtttgtgaactctcagtatgataggctccaagctgataccaacatagctatgattcatgctgcagacaaacgcgttcatagcattcgggaagcttaccttcctgaacttagcgtgattccgggtgtcaatgctgctatctttgaagagttagaagggcgcatcttcactgcattctccttgtatgatgcgaggaatgtcatcaagaatggtgacttcaacaatggcctatcctgctggaatgtgaaagggcacgtagatgtagaagaacagaacaatcaccgctctgtccttgttgttcctgagtgggaagcagaagtttcacaagaagttcgtgtctgtcctggtcgtggctacattcttcgtgttaccgcgtacaaagaaggatacggagaaggttgcgtcaccatacacgagattgagaacaacaccgacgagctgaagttcagcaactgcgtcgaggaggaagtctacccaaacaacaccgtaacttgcaatgactacactgcgactcaagaggagtatgagggtacttacacttctcgcaatcgaggatacgatggagcctatgagagcaactcttctgtacccgctgactatgcatcagcctatgaggagaaggcttacaccgatggacgtagggacaatccttgcgaatctaacagaggctatggggactacacaccgttaccagccggctatgtcaccaaagagttagagtactttccagaaaccgacaaggtttggattgagattggagaaacggaaggaacattcattgttgatagcgtggagttacttctgatggaggaatgagtagttagcttaatcacctagagctcggttacctatcaaaatctatttagaaatacacaatattttgttgcaggcttgctggagaatcgatctgctatcataaaaattacaaaaaaattttatttgcctcaattattttaggattggtattaaggacgcttaaattatttgtcgggtcactacgcatcattgtgattgagaagatcagcgatacgaaatattcgtagtactatcgataatttatttgaaaattcataagaaaagcaaacgttacatgaattgatgaaacaatacaaagacagataaagccacgcacatttaggatattggccgagattactgaatattgagtaagatcacggaatttctgacaggagcatgtcttcaattcagcccaaatggcagttgaaatactcaaaccgccccatatgcaggagcggatcattcattgtttgtttggttgcctttgccaacatgggagtccaaggttgcggccgcgcgccgacccagctttcttgtacaaagtggttgcggccgcttaattaaatttaaatgcccgggcgtttaaacgcggccgcttaattaaggccggcctgcagcaaacccagaaggtaattatccaagatgtagcatcaagaatccaatgtttacgggaaaaactatggaagtattatgtaagctcagcaagaagcagatcaatatgcggcacatatgcaacctatgttcaaaaatgaagaatgtacagatacaagatcctatactgccagaatacgaagaagaatacgtagaaattgaaaaagaagaaccaggcgaagaaaagaatcttgaagacgtaagcactgacgacaacaatgaaaagaagaagataaggtcggtgattgtgaaagagacatagaggacacatgtaaggtggaaaatgtaagggcggaaagtaaccttatcacaaaggaatcttatcccccactacttatccttttatatttttccgtgtcatttttgcccttgagttttcctatataaggaaccaagttcggcatttgtgaaaacaagaaaaaatttggtgtaagctattttctttgaagtactgaggatacaacttcagagaaatttgtaagtttgtagatctccatgtctccggagaggagaccagttgagattaggccagctacagcagctgatatggccgcggtttgtgatatcgttaaccattacattgagacgtctacagtgaactttaggacagagccacaaacaccacaagagtggattgatgatctagagaggttgcaagatagatacccttggttggttgctgaggttgagggtgttgtggctggtattgcttacgctgggccctggaaggctaggaacgcttacgattggacagttgagagtactgtttacgtgtcacataggcatcaaaggttgggcctaggatccacattgtacacacatttgcttaagtctatggaggcgcaaggttttaagtctgtggttgctgttataggccttccaaacgatccatctgttaggttgcatgaggctttgggatacacagcccggggtacattgcgcgcagctggatacaagcatggtggatggcatgatgttggtttttggcaaagggattttgagttgccagctcctccaaggccagttaggccagttacccagatctgaggtaccctgagcttgagcttatgagcttatgagcttagagctcggatccactagtaacggccgccagtgtgctggaattcgcccttgactagataggcgcccagatcggcggcaatagcttcttagcgccatcccgggttgatcctatctgtgttgaaatagttgcggtgggcaaggctctctttcagaaagacaggcggccaaaggaacccaaggtgaggtgggctatggctctcagttccttgtggaagcgcttggtctaaggtgcagaggtgttagcgggatgaagcaaaagtgtccgattgtaacaagatatgttgatcctacgtaaggatattaaagtatgtattcatcactaatataatcagtgtattccaatatgtactacgatttccaatgtctttattgtcgccgtatgtaatcggcgtcacaaaataatccccggtgactttcttttaatccaggatgaaataatatgttattataatttttgcgatttggtccgttataggaattgaagtgtgcttgcggtcgccaccactcccatttcataattttacatgtatttgaaaaataaaaatttatggtattcaatttaaacacgtatacttgtaaagaatgatatcttgaaagaaatatagtttaaatatttattgataaaataacaagtcaggtattatagtccaagcaaaaacataaatttattgatgcaagtttaaattcagaaatatttcaataactgattatatcagctggtacattgccgtagatgaaagactgagtgcgatattatggtgtaatacatagcggccgggtttctagtcaccggttaggatccgtttaaactcgaggctagcgcatgcacatagacacacacatcatctcattgatgcttggtaataattgtcattagattgtttttatgcatagatgcactcgaaatcagccaattttagacaagtatcaaacggatgtgacttcagtacattaaaaacgtccgcaatgtgccattggcaacaacctctgatgccgtaacttttctttgttggttcagaaatccaaccgttatggataattctaaatcctcatacttcatctttccacaaaagcacaaattctcctactagtaggctttagatgtgttttatatctctaaaagcattaaatattttttatttttcattcattatttcataaaagatagtaaagtcccctttgtctgcagagaaaatggtgaaaaaagaaaataaataaataaataataaagtgatgtaacattcatatttttatattatattttaattcaaaaactttaatctcatgtgacttttatttttcttttcactaccgaacggagcctgagagaatatagcattactcaaccgttatattgctgaaaaatttctagtaatgaccatttgaatttctcgagagcttccgttgttcaatttctagcgtctctatatgtgatgcggcagaatcggacctccgagtgaaaagttatgaccatttgaatttttcgaaagcttccgttgtttaatttcgagcgtctcgatatattatgcggctgaatcggacctccgagtgaaaagttatgatcatttgaattgctcaagagcttccattgttcaatttcgaacgtctcgatatattatgcgcatgaatcagacatccgagtgaaaagttatgaccatttgaattgctcaagagtttccattgccccattttgaacgtctcgatatattatgcgcctgaatcggacttccgagttaaatgttattctcaagagcttttgttgttcaatttcaagcgtctcgatatattatgcacctgaatcggatctccgagtgaaatgttagttccatttgaattggtcaagtgcttccatagcatggtgggcgagagtaccaccctccaccaaacaaacccactctctatattcctatttctgtatacttctctagacaacgttagtagtaacacaaccactctcattagccttaaccgacccagagaaaacacgcatcggttaatgctattcctttctctgaaatcgcttcgaagacaagaaaagaattaataaccaaaagaaaccgcacctcataccagaaatagcttacatgcctaacgattttctttgcttttaa

SEQ ID NO: 29 - DNA, 15294 bp, Artificial Sequence
  Expected sequence of soybean event 9582.814.19.1
ttaacaatgaccaagatttatgctatatagaagacttggagggcttaaggctatgatatattatggatgatatggttctgatttgtgtagtttcgaaggatcaaatcaaccatttgttggtacaatgggaagaaaaaatgttttcatcattccactctattgaaaaagatccaacaattgtaacaccccgacgaatcacaccggaaagagaagaatccaaagattgtgtaggtatgagactgtatagttgatgaaaacttaaaaaaattaattggtactacttataccaacaagatgcatatatttttcgatagcctatcacataagaacttcatagttaagggtgcttaacttggagtagttatgaaatgagtgaccttttaaaataattattgtcttaggttattgtatgaaaataaaaaataataataaatatacataaaaaataataattttataaaattaaccttatattatcattaatttatttttagattttgttattcattattaatatatgaggtataaatgaaaaatataattaatgtcacattaaaaaattaaaatgataattattttgaaacaaattatttatttttatacgacaattataatagaaatttgagagtaaaaaaaaattgaaaattcataaaatatatgaatatattcatttctcctatccgtcaaataaatctgctccataatttatctaagcattggtcttgtagttcagagtaataaaattttagcaattattagttagtacagatacatttaaagaaataatatattttagcaactagaagtttataaaaagttttaaattataaagacttatatataaatttagtaaaactagatggatgtcccaagtaatttttatataactattctcgtacaacattaatgaaaatcttgtttctattatttatatgtatattattattttattttggaacaatatgggattaaaaactcttataaattaaatcttagaataagttttcctaacatgttttttttatggatgttttcctaacatgtttggttatcttagttttgctttaattttgtcggattatttttggactttattaggtaattttgataaaacttttagttgatgttagtagtttactcttacataatgatttgatattgaatgtgtataattggaaggcaataaatgaagatcaagcgtacaagagttcgccaatcaagaggatttgaagagagtaaaatattatgcgaagtcccatgtgaagaaaatccaaccattggaataaaaaataaagttttttctttggaattgctaatgctacagcacttattggtacttgtcctaaaaatgaaactctagctatatttagcacttgatattcatgaatcaaacttctctatgaaataaccgcggtgcgcatcggtgcctgttgatcccgcgcaagttgggatcttgaagcaagttccgctcatcactaagtcgcttagcatgtttgaccttctcggacaactccttcttctctttaattgatcaacagtcagcatcatcacaccaaaagttaggcccgaatagtttgaaattagaaagctcgcaattgaggtctacaggccaaattcgctcttagccgtacaatattactcaccggatcctaaccggtgtgatcatgggccgcgattaaaaatctcaattatatttggtctaatttagtttggtattgagtaaaacaaattcggcgccatgcccgggcaagcggccgcacaagtttgtacaaaaaagcaggctccgcggtgactgactgaaaagcttgtcgacctgcaggtcaacggatcaggatattcttgtttaagatgttgaactctatggaggtttgtatgaactgatgatctaggaccggataagttcccttcttcatagcgaacttattcaaagaatgttttgtgtatcattcttgttacattgttattaatgaaaaaatattattggtcattggactgaacacgagtgttaaatatggaccaggccccaaataagatccattgatatatgaattaaataacaagaataaatcgagtcaccaaaccacttgccttttttaacgagacttgttcaccaacttgatacaaaagtcattatcctatgcaaatcaataatcatacaaaaatatccaataacactaaaaaattaaaagaaatggataatttcacaatatgttatacgataaagaagttacttttccaagaaattcactgattttataagcccacttgcattagataaatggcaaaaaaaaacaaaaaggaaaagaaataaagcacgaagaattctagaaaatacgaaatacgcttcaatgcagtgggacccacggttcaattattgccaattttcagctccaccgtatatttaaaaaataaaacgataatgctaaaaaaatataaatcgtaacgatcgttaaatctcaacggctggatcttatgacgaccgttagaaattgtggttgtcgacgagtcagtaataaacggcgtcaaagtggttgcagccggcacacacgagtcgtgtttatcaactcaaagcacaaatacttttcctcaacctaaaaataaggcaattagccaaaaacaactttgcgtgtaaacaacgctcaatacacgtgtcattttattattagctattgcttcaccgccttagctttctcgtgacctagtcgtcctcgtcttttcttcttcttcttctataaaacaatacccaaagcttcttcttcacaattcagatttcaatttctcaaaatcttaaaaactttctctcaattctctctaccgtgatcaaggtaaatttctgtgttccttattctctcaaaatcttcgattttgttttcgttcgatcccaatttcgtatatgttctttggtttagattctgttaatcttagatcgaagacgattttctgggtttgatcgttagatatcatcttaattctcgattagggtttcataaatatcatccgatttgttcaaataatttgagttttgtcgaataattactcttcgatttgtgatttctatctagatctggtgttagtttctagtttgtgcgatcgaatttgtcgattaatctgagtttttctgattaacagagatctccatggagaacaatatccagaaccagtgtgtcccatacaattgcctcaacaatcctgaagttgagatcctcaacgaagagaggagcactggacgccttccccttgacatctccctctccctcacaaggttccttttgtctgagtttgttcctggtgtgggtgtggcctttggcctctttgacctcatctggggcttcatcaccccatctgattggagcctcttccttctccagattgaacaattgattgagcagaggattgagacccttgaaaggaacagagccatcaccacacttcgtggccttgctgacagctatgaaatctacattgaagcactccgtgagtgggaagccaatcccaacaatgctcaactccgtgaagatgtgaggattcgctttgccaacacagatgacgctttgatcacagccatcaacaatttcaccctcaccagctttgagatccctttgctctcagtctatgttcaagctgcaaacctccacttgagcttgcttagggatgctgtgtccttcggacaaggttggggacttgacatagccactgtcaacaatcactacaacagactcatcaacttgattcatcgctacaccaaacattgcttggacacctacaatcaaggattggagaacctcagaggcaccaacactcgccaatgggcaaggttcaaccagtttagaagggatctcacactcactgtgcttgacatagttgctctcttccccaactatgatgttcgcacctacccaattcaaaccagctcccaacttacaagggaaatctacacctcctcagtcattgaggacagcccagtttctgccaacatacccaatggtttcaaccgtgctgagtttggtgtcagaccaccccatctcatggacttcatgaactccttgtttgtgactgccgagactgttaggtcccaaactgtgtggggaggccaccttgttagctcccgcaacaccgctggcaaccgcatcaacttcccatcctatggggttttcaatcctggtggagccatctggattgcagatgaggacccaaggcctttctacagaaccttgtcagatcctgtctttgtcagaggaggctttggcaatccacactatgttcttggtttgaggggagtggcttttcagcagactggcaccaatcacacccgcacattcagaaacagcggcaccattgacagccttgatgagatcccacctcaagacaacagcggagcaccctggaacgactactcccatgtgctcaatcatgtcacctttgtgcgctggcctggtgagatcagcggttcagattcttggagagcaccaatgttctcatggacccatcgctctgccacacccacaaacaccattgatccagagagaatcacccagattcccttggtgaaggcacacacacttcagtctggaaccacagttgtcagagggcctgggttcactggtggagacattctcagacgcacctctggagggccatttgcttacaccattgtcaacatcaatgggcaacttccccagcgttaccgtgccagaatccgctatgcttccaccactaacttgagaatctatgtcacagttgctggtgaaaggatctttgctggtcagttcaacaagacaatggacactggtgatccattgacattccagtcattctcctatgccaccatcaacactgcattcacctttccaatgagccagtccagcttcacagtgggtgcagataccttcagctccggcaatgaggtgtacattgaccgctttgagttgattccagtgactgccacacttgaggctgagtctgacttggagcgtgctcagaaggccgtgaatgctctcttcacctcttcaaatcagattgggctcaagacagatgtgactgactaccatatagaccgtgtttccaatcttgttgagtgcctctctgatgagttctgcttggatgagaagaaagagttgtcagagaaggtcaagcacgccaagaggctctctgatgagaggaacttgcttcaagatcccaacttcagagggatcaaccgtcaattggatcgtggatggaggggatcaactgacataaccattcaaggaggtgacgatgtgttcaaggagaactatgtcacactcttggggacctttgatgagtgctacccaacatacctttaccagaagatagacgaaagcaagctcaaggcctacacaagataccagttgagaggttacattgaggactctcaagaccttgaaatctacctcatcagatacaacgccaaacatgagacagtcaatgtgcctgggactggttcactctggccactttcagccccaagccccattggcaagtgtgcccatcactcacatcacttctccttggacatagatgttggctgcactgacttgaatgaggaccttggtgtgtgggtgatcttcaagatcaagacccaagatggccatgcaaggttgggcaatcttgagtttcttgaagagaaaccacttgttggagaagcccttgccagagtgaagagggctgagaagaaatggagggacaagagagagaagttggagtgggaaacaaacattgtgtacaaagaagccaaagaatcagttgatgctttgtttgtgaactcccaatatgataggctccaagctgacaccaacatagcaatgattcatgctgcagacaaaagggttcacagcattcgtgaagcataccttcctgaactctcagtgattcctggggtcaatgctgcaatctttgaagagcttgaaggacgcatcttcactgccttctccttgtatgatgcaaggaatgtcatcaagaatggtgacttcaacaatggcctttcctgctggaatgtgaaagggcacgtggatgttgaagagcagaacaatcaccgctctgtccttgttgtccctgagtgggaagctgaagtttcacaagaagttcgtgtctgccctggtcgtggctacattcttcgtgtgactgcttacaaagaaggctatggagaaggttgtgtcaccatccacgagatagagaacaatactgatgaattgaagttcagcaactgtgttgaggaagaggtctacccaaacaatactgtcacttgcaatgactacactgcaactcaagaagagtatgagggcacttacacttctcgcaaccgtggctatgatggagcctatgagagcaactcatctgtgcctgctgactatgcttcagcctatgaagagaaggcatacactgatggaaggcgtgacaatccttgtgaaagcaacagaggctatggggactacacacccctcccagctggctatgtgaccaaagagttggagtactttcctgaaactgacaaggtttggattgagataggagaaactgaaggcacattcatagttgactctgtggagcttttgctcatggaagagtgagtagttagcttaatcacctagagctcggtcaccagcataatttttattaatgtactaaattactgttttgttaaatgcaattttgctttctcgggattttaatatcaaaatctatttagaaatacacaatattttgttgcaggcttgctggagaatcgatctgctatcataaaaattacaaaaaaattttatttgcctcaattattttaggattggtattaaggacgcttaaattatttgtcgggtcactacgcatcattgtgattgagaagatcagcgatacgaaatattcgtagtactatcgataatttatttgaaaattcataagaaaagcaaacgttacatgaattgatgaaacaatacaaagacagataaagccacgcacatttaggatattggccgagattactgaatattgagtaagatcacggaatttctgacaggagcatgtcttcaattcagcccaaatggcagttgaaatactcaaaccgccccatatgcaggagcggatcattcattgtttgtttggttgcctttgccaacatgggagtccaaggttgcggccgcgcgccgaaaacaactttgtatacaaaagttgccgcggtgactgactgaactaaacccagaaggtaattatccaagatgtagcatcaagaatccaatgtttacgggaaaaactatggaagtattatgtaagctcagcaagaagcagatcaatatgcggcacatatgcaacctatgttcaaaaatgaagaatgtacagatacaagatcctatactgccagaatacgaagaagaatacgtagaaattgaaaaagaagaaccaggcgaagaaaagaatcttgaagacgtaagcactgacgacaacaatgaaaagaagaagataaggtcggtgattgtgaaagagacatagaggacacatgtaaggtggaaaatgtaagggcggaaagtaaccttatcacaaaggaatcttatcccccactacttatccttttatatttttccgtgtcatttttgcccttgagttttcctatataaggaaccaagttcggcatttgtgaaaacaagaaaaaatttggtgtaagctattttctttgaagtactgaggatacaacttcagagaaatttgtaagtttgtagatccaacaatggacaacaatcccaacatcaacgagtgcattccttacaactgcctgagcaaccctgaggttgaggtgctgggtggagaacggattgagactggttacacacctatcgacatctcgttgtcacttacccaattccttttgtcagagttcgtgcccggtgctggattcgtgcttggacttgtcgatatcatttggggaatctttggtccctctcaatgggacgcctttcttgtacagatagagcagttaattaaccaaagaatagaagaattcgctaggaaccaagccatctcaaggttagaaggcctcagcaacctttaccagatttacgcagaatcttttcgagagtgggaagcagacccgaccaatcctgccttaagagaggagatgcgcattcaattcaatgacatgaacagcgcgctgacgaccgcaattccgctcttcgccgttcagaattaccaagttcctcttttatccgtgtacgtgcaggctgccaacctgcacttgtcggtgctccgcgatgtctccgtgttcggacaacggtggggctttgatgccgcaactatcaatagtcgttataatgatctgactaggcttattggcaactataccgattatgctgttcgctggtacaacacgggtctcgaacgtgtctggggaccggattctagagattgggtcaggtacaaccagttcaggcgagagttgacactaactgtcctagacattgtcgctctctttcccaactacgactctaggcgctacccaatccgtactgtgtcacaattgacccgggaaatctacacaaacccagtcctcgagaacttcgacggtagctttcgaggctcggctcagggcatagagagaagcatcaggtctccacacctgatggacatattgaacagtatcacgatctacaccgatgcgcaccgcggttattactactggtcagggcatcagatcatggcatcacccgttgggttctctggaccagaattcactttcccactttacgggactatgggcaatgcagctccacaacaacgtattgttgctcaactcggtcagggcgtgtatagaaccttgtccagcactctatataggagacctttcaacatcggcatcaacaatcaacaattgtctgtgcttgacgggacagaatttgcctatggaacctcctcaaatctgccatccgctgtctacagaaagagcggaacagttgatagcttggatgagatccctccacagaacaacaacgttccacctaggcaagggtttagccatcgccttagccatgtgtccatgttccgttcaggctttagtaatagcagcgttagtatcatcagagctccgatgttctcttggatacatcgtagtgctgagtttaacaacataattgcatccgatagcattactcagatcccagctgtcaaggggaactttctctttaatggttctgtcatttcaggaccaggattcactggaggcgacttggttaggctgaattcttccggcaacaacatccagaatagagggtatattgaagtgcccattcacttcccatcgacatctaccagatatcgtgttcgtgtaaggtatgcctctgttacccctattcacctcaacgtcaattggggtaattcctccatcttttccaatacagtaccagcgacagctacatccttggataatctccaatctagcgatttcggttacttcgaaagtgccaatgccttcacctcttccctaggtaacatagtaggtgttagaaatttctccggaaccgccggagtgataatcgaccgcttcgaattcattcccgttactgcaacgctcgaggcagagtctgacttggaaagagcacagaaggcggtgaatgctctgttcacttcgtccaatcagattgggctcaagacagatgtgactgactatcacatcgatcgcgtttccaaccttgttgagtgcctctctgatgagttctgtttggatgagaagaaggagttgtccgagaaggtcaaacatgctaagcgacttagtgatgagcggaacttgcttcaagatcccaactttcgcgggatcaacaggcaactagatcgtggatggaggggaagtacggacatcaccattcaaggaggtgatgatgtgttcaaggagaactatgttacgctcttgggtacctttgatgagtgctatccaacatacctgtaccagaagatagatgaatcgaaactcaaagcctacacaagataccagttgagaggttacatcgaggacagtcaagaccttgagatctacctcatcagatacaacgccaaacatgagacagtcaatgtgcctgggacgggttcactctggccactttcagccccaagtcccatcggcaagtgtgcccatcactcacaccacttctccttggacatagacgttggctgtaccgacctgaacgaagacctcggtgtgtgggtgatcttcaagatcaagactcaagatggccatgccaggctaggcaatctggagtttctagaagagaaaccacttgttggagaagccctcgctagagtgaagagggctgagaagaagtggagggacaagagagagaagttggaatgggaaacaaacattgtgtacaaagaagccaaagaaagcgttgacgctctgtttgtgaactctcagtatgataggctccaagctgataccaacatagctatgattcatgctgcagacaaacgcgttcatagcattcgggaagcttaccttcctgaacttagcgtgattccgggtgtcaatgctgctatctttgaagagttagaagggcgcatcttcactgcattctccttgtatgatgcgaggaatgtcatcaagaatggtgacttcaacaatggcctatcctgctggaatgtgaaagggcacgtagatgtagaagaacagaacaatcaccgctctgtccttgttgttcctgagtgggaagcagaagtttcacaagaagttcgtgtctgtcctggtcgtggctacattcttcgtgttaccgcgtacaaagaaggatacggagaaggttgcgtcaccatacacgagattgagaacaacaccgacgagctgaagttcagcaactgcgtcgaggaggaagtctacccaaacaacaccgtaacttgcaatgactacactgcgactcaagaggagtatgagggtacttacacttctcgcaatcgaggatacgatggagcctatgagagcaactcttctgtacccgctgactatgcatcagcctatgaggagaaggcttacaccgatggacgtagggacaatccttgcgaatctaacagaggctatggggactacacaccgttaccagccggctatgtcaccaaagagttagagtactttccagaaaccgacaaggtttggattgagattggagaaacggaaggaacattcattgttgatagcgtggagttacttctgatggaggaatgagtagttagcttaatcacctagagctcggttacctatcaaaatctatttagaaatacacaatattttgttgcaggcttgctggagaatcgatctgctatcataaaaattacaaaaaaattttatttgcctcaattattttaggattggtattaaggacgcttaaattatttgtcgggtcactacgcatcattgtgattgagaagatcagcgatacgaaatattcgtagtactatcgataatttatttgaaaattcataagaaaagcaaacgttacatgaattgatgaaacaatacaaagacagataaagccacgcacatttaggatattggccgagattactgaatattgagtaagatcacggaatttctgacaggagcatgtcttcaattcagcccaaatggcagttgaaatactcaaaccgccccatatgcaggagcggatcattcattgtttgtttggttgcctttgccaacatgggagtccaaggttgcggccgcgcgccgacccagctttcttgtacaaagtggttgcggccgcttaattaaatttaaatgcccgggcgtttaaacgcggccgcttaattaaggccggcctgcagcaaacccagaaggtaattatccaagatgtagcatcaagaatccaatgtttacgggaaaaactatggaagtattatgtaagctcagcaagaagcagatcaatatgcggcacatatgcaacctatgttcaaaaatgaagaatgtacagatacaagatcctatactgccagaatacgaagaagaatacgtagaaattgaaaaagaagaaccaggcgaagaaaagaatcttgaagacgtaagcactgacgacaacaatgaaaagaagaagataaggtcggtgattgtgaaagagacatagaggacacatgtaaggtggaaaatgtaagggcggaaagtaaccttatcacaaaggaatcttatcccccactacttatccttttatatttttccgtgtcatttttgcccttgagttttcctatataaggaaccaagttcggcatttgtgaaaacaagaaaaaatttggtgtaagctattttctttgaagtactgaggatacaacttcagagaaatttgtaagtttgtagatctccatgtctccggagaggagaccagttgagattaggccagctacagcagctgatatggccgcggtttgtgatatcgttaaccattacattgagacgtctacagtgaactttaggacagagccacaaacaccacaagagtggattgatgatctagagaggttgcaagatagatacccttggttggttgctgaggttgagggtgttgtggctggtattgcttacgctgggccctggaaggctaggaacgcttacgattggacagttgagagtactgtttacgtgtcacataggcatcaaaggttgggcctaggatccacattgtacacacatttgcttaagtctatggaggcgcaaggttttaagtctgtggttgctgttataggccttccaaacgatccatctgttaggttgcatgaggctttgggatacacagcccggggtacattgcgcgcagctggatacaagcatggtggatggcatgatgttggtttttggcaaagggattttgagttgccagctcctccaaggccagttaggccagttacccagatctgaggtaccctgagcttgagcttatgagcttatgagcttagagctcggatccactagtaacggccgccagtgtgctggaattcgcccttgactagataggcgcccagatcggcggcaatagcttcttagcgccatcccgggttgatcctatctgtgttgaaatagttgcggtgggcaaggctctctttcagaaagacaggcggccaaaggaacccaaggtgaggtgggctatggctctcagttccttgtggaagcgcttggtctaaggtgcagaggtgttagcgggatgaagcaaaagtgtccgattgtaacaagatatgttgatcctacgtaaggatattaaagtatgtattcatcactaatataatcagtgtattccaatatgtactacgatttccaatgtctttattgtcgccgtatgtaatcggcgtcacaaaataatccccggtgactttcttttaatccaggatgaaataatatgttattataatttttgcgatttggtccgttataggaattgaagtgtgcttgcggtcgccaccactcccatttcataattttacatgtatttgaaaaataaaaatttatggtattcaatttaaacacgtatacttgtaaagaatgatatcttgaaagaaatatagtttaaatatttattgataaaataacaagtcaggtattatagtccaagcaaaaacataaatttattgatgcaagtttaaattcagaaatatttcaataactgattatatcagctggtacattgccgtagatgaaagactgagtgcgatattatggtgtaatacatagcggccgggtttctagtcaccggttaggatccgtttaaactcgaggctagcgcatgcacatagacacacacatcatctcattgatgcttggtaataattgtcattagattgtttttatgcatagatgcactcgaaatcagccaattttagacaagtatcaaacggatgtgacttcagtacattaaaaacgtccgcaatatgatattcattaattttatattatctaaaagagttaaaagagaaaaaagaaatatgacaatttttttctttcacatcttctaacctaaaagtatgactctatggaggctaagtttagaaaaagatacggatctagggtgtggaaacatcaatggtcaactccttttatatttcaatcaattgggttttgctttatctttacattttctccttttattttccacgtctattcaaatctacttgttagcgggtgattactcttttttcttttatagatgccaattatttctctcctatgtattaaattagagtatattgtcttgaaagtgacttagtattttagtttatagtctcttaaagaacgacaccttttattcttaactctctttatcaagttttaatttaaaattattttaaattaagtatgcatacatatcttaatatttttcttaattatttttaaattccctaaatttaatgttttcatacaatgtaagagatatacatattaattatatttaaagataaaacttactttcctgcaataaaataaagaaaaggacagtcatacaattatataattaatccagaatatttatagcttttaaacatttattttctatcaattaagtaataactttaaataaaattaagagtacttttttatactccaaagaatttatttattttcaacaaaatcgtctgactgtttcaattgatcattatcagcctagcataacctaaatttcattttcaaacataacttttggcaccaaatcacccggcattgcaaaaaagtcttttgcgatatgaccctccacgacgcagaaccactgttattcattaccatcacttttaatcctaatttcccatacacttaccctttccatgacatcttcaaagcctttattttgcttttcttgtttaagctgttttaacctaatttcatgcatataaacaaagagtaaagcaaaggcaaatatttgtacgtatagtttttagacagaaaaggaaagtaaattatagagataatgaagtttgctcttttaaattcgtcgtgatgttatccatcatatctaaatgcttattcctgtttttgtcttttttctcttttaccggagtttattttatataattaattaaagttagtagatctatattctttttcatagataatccatcttctttggaggcacatcgatcattaatcatagagttttgagaagcattatcactaaagcttcaattaattatatccaataaacggtattggtgtatgatgttatgatagcaaatagataatctaatctatacgagccacaaaaggggcatgaactctatctcgaagaaattggagatgaagggattgagattggcaccttgtgctattattgcccactaatcatt